European Patent Application EP 4 480 510 A1, published December 25, 2024. Title: BIOABSORBABLE AND PHOTOCURABLE COMPOSITION, BIOABSORBABLE GUIDED TISSUE REGENERATION COMPOSITION, AND GRAFTING METHOD USING THE SAME. Applicant: NIBEC Co., Ltd. The sequence listing filed with the application follows.

SEQUENCE LISTING (5 sequences)

SEQ ID NO: 1 - protein, 15 aa, synthetic construct
  REGION 1..15: note = PEPTIDE HAVING ANTIBACTERIAL, ANTIINFLAMMATION OR TISSUE REGENERATION
GKCSTRGRKSSRRKK

SEQ ID NO: 2 - protein, 22 aa, synthetic construct
  REGION 1..22: note = PEPTIDE HAVING ANTIBACTERIAL, ANTIINFLAMMATION OR TISSUE REGENERATION
CPRRYKQIGTCGLPGTKCCKKP

SEQ ID NO: 3 - protein, 15 aa, synthetic construct
  REGION 1..15: note = PEPTIDE HAVING ANTIBACTERIAL, ANTIINFLAMMATION OR TISSUE REGENERATION
GKCSTRGRKCCRRKK

SEQ ID NO: 4 - protein, 18 aa, synthetic construct
  REGION 1..18: note = PEPTIDE HAVING ANTIBACTERIAL, ANTIINFLAMMATION OR TISSUE REGENERATION
RKIEIVRKKPIFKKATVT

SEQ ID NO: 5 - protein, 22 aa, synthetic construct
  REGION 1..22: note = PEPTIDE HAVING ANTIBACTERIAL, ANTIINFLAMMATION OR TISSUE REGENERATION
CKRKKKGKGLGKKRDPCLRKYK